European Patent Application EP 4 477 734 A2, published December 18, 2024. Title: PROTEASE VARIANTS AND POLYNUCLEOTIDES ENCODING SAME. Applicant: Novozymes A/S. Application EP. The sequence listing filed with the application follows.

SEQUENCE LISTING (3 sequences)

SEQ ID NO: 1 - DNA, 1263 bp, bacillius sp.
  sig_peptide 1..80
  mat_peptide 331..1263
  source 1..1263: mol_type = genomic DNA
  CDS 1..1263
atgaagaaaccgttggggaaaattgtcgcaagcaccgcactactcatttctgttgcttttagttcatcgatcgcatcggctgcacttgcaaaagacaaagttgaggtaaaggaacaagattcatatcgtgtgctaatcaaagcaccaactacatcaatcagtacttttcaatcacaatacgatgtccgttgggattttggcaaagagggatttacaacagatgttgatgccaaacagctccaaacgcttcaaagcaacaaagacattcaaattcagaaggtaaatgaaatgacagtagaaactgttacaacagaaaaggcggaagtgacggcggtaccaagtacacaaaccccttggggcataaagtcaatttataatgatcaatcaattacaaaaacaactggaggcagcggaattaaggtagctgttttagatacaggggtttatacaagccatttagatttagctggttctgccgagcaatgcaaggattttacccaatctaatcctttagtagatggttcatgcaccgatcgccaagggcatggtacacatgttgccggaactgtattggcgcatggaggcagtaatggacaaggcgtttacggggtggctccgcaagcgaaactatgggcatataaagtattaggagataacggcagcggatactctgatgatattgcagcagctatcagacatgtagctgatgaagcttcacgtacaggttccaaagtagtaattaatatgtcgctaggttcatctgccaaggattcattgattgctagtgcagtagattatgcatatggaaaaggtgtattaatcgttgctgcggctggtaatagtgggtcaggcagcaatacaatcggctttcctggcgggcttgtaaatgcagtggcagtagcggcattggagaatgttcagcaaaatggaacttatcgagtagctgatttctcatctagagggaatccggcaactgctggagattatatcattcaagagcgtgatattgaagtttcagctccgggagcaagtgtagagtctacatggtacactggcggttataatacgatcagcggtacatcaatggctacacctcatgtagctgggttagctgctaaaatctggtcagcgaatacttcattaagtcatagccaactgcgcacagaattgcaaaatcgcgctaaagtatatgatattaaaggtggtatcggagccggaacaggtgacgattatgcatcagggttcggatatccaagagtaaaa

SEQ ID NO: 2 - protein, 421 aa, bacillius sp.
MKKPLGKIVASTALLISVAFSSSIASAALAKDKVEVKEQDSYRVLIKAPTTSISTFQSQYDVRWDFGKEGFTTDVDAKQLQTLQSNKDIQIQKVNEMTVETVTTEKAEVTAVPSTQTPWGIKSIYNDQSITKTTGGSGIKVAVLDTGVYTSHLDLAGSAEQCKDFTQSNPLVDGSCTDRQGHGTHVAGTVLAHGGSNGQGVYGVAPQAKLWAYKVLGDNGSGYSDDIAAAIRHVADEASRTGSKVVINMSLGSSAKDSLIASAVDYAYGKGVLIVAAAGNSGSGSNTIGFPGGLVNAVAVAALENVQQNGTYRVADFSSRGNPATAGDYIIQERDIEVSAPGASVESTWYTGGYNTISGTSMATPHVAGLAAKIWSANTSLSHSQLRTELQNRAKVYDIKGGIGAGTGDDYASGFGYPRVK

SEQ ID NO: 3 - protein, 311 aa, Bacillus sp. [sequence omitted]